European Patent Application EP 4 458 843 A1, published November 6, 2024. Title: mRNA vaccine. Applicant: 广州国家实验室. Application WO PCT/CN2022/144148, filed December 30, 2022. The sequence listing filed with the application follows.

SEQUENCE LISTING (10 sequences)

SEQ ID NO: 1 - RNA, 1299 nt, synthetic construct
  source 1..1299: mol_type = other RNA
  misc_feature 1..1299: note = n is 1-methyl-3'-pseudouridylyl
anggagacagacacacnccngcnangggnacngcngcncngggnnccaggnnccacnggngaccgnacgngngancngccncagacncanncccngggnagnaggagaacccngangcngcnggcacaaangagaaaaancncacngnnnagnngccngaaggancgacacgacnnngggnnnccccaagaagagnnnggcaaccaannccagaaagcagagacaancccngncnngcacgaganganccagcaaancnnnaaccngnnnncnaccaaagannccnccgccgcangggangagacccngcncgacaagnnnnanacngaacngnancagcagcngaacgannnggaggcgngcgnganncagggcgnnggggnnaccgaaaccccncngangaaggaagacncnanannggcngnnaggaagnannnncagagaancaccnngnannngaaagagaagaagnacagnccangngcnngggaggnngnccgggccgaaancangagaagnnncagcnngncaacnaaccngcaggaaagccncaggagcaaggaanncgaaggcggnggaggcagcggaggcggnggcagcggnggcggaggcagcncnagaagggngcagcccaccgagagcancgngaggnnccccaacancaccaaccngngccccnncggcgaggngnncaacgccaccaggnncgccagcgngnacgccnggaacaggaagaggancagcaacngcgnggccgacnacagcgngcngnacaacagcgccagcnncagcaccnncaagngcnacggcgngagccccaccaagcngaacgaccngngcnncaccaacgngnacgccgacagcnncgngancaggggcgacgaggngaggcagancgcccccggccagaccggcaagancgccgacnacaacnacaagcngcccgacgacnncaccggcngcgngancgccnggaacagcaacaaccnggacagcaaggngggcggcaacnacaacnaccngnacaggcngnncaggaagagcaaccngaagcccnncgagagggacancagcaccgagancnaccaggccggcagcacccccngcaacggcgnggagggcnncaacngcnacnncccccngcagagcnacggcnnccagcccaccaacggcgngggcnaccagcccnacagggnggnggngcngagcnncgagcngcngcacgcccccgccaccgngngcggccccaagaagagcaccaaccnggngaagaacaagngcgngaacnnncncgagnag

SEQ ID NO: 2 - RNA, 1185 nt, synthetic construct
  source 1..1185: mol_type = other RNA
  misc_feature 1..1185: note = n is 1-methyl-3'-pseudouridylyl
anggagacagacacacnccngcnangggnacngcngcncngggnnccaggnnccacnggngaccgnacggcaccngcnagancaccancnccnncaacacagccnngggaacacgnnaacgccanncaggaggcncggcgcnngcngaancngagcaggganacagccgcagagangaacgaaacagnggaagngannagngaaangnnngaccnncaagagccaacangccngcagaccagacnngagcngnacaagcaggggcngaggggancncnnacaaaacngaaagggccacnnaccanganggccncacacnanaaacagcacngcccnccaacaccngagacgnccngngcnacncagannancacnnncgagagcnnnaaagaaaancngaaggacnnncnccnggnganccccnncganngcngggagccngnccaggagnncgaaggcggnggaggcagcggaggcggnggcagcggnggcggaggcagcncnagaagggngcagcccaccgagagcancgngaggnnccccaacancaccaaccngngccccnncggcgaggngnncaacgccaccaggnncgccagcgngnacgccnggaacaggaagaggancagcaacngcgnggccgacnacagcgngcngnacaacagcgccagcnncagcaccnncaagngcnacggcgngagccccaccaagcngaacgaccngngcnncaccaacgngnacgccgacagcnncgngancaggggcgacgaggngaggcagancgcccccggccagaccggcaagancgccgacnacaacnacaagcngcccgacgacnncaccggcngcgngancgccnggaacagcaacaaccnggacagcaaggngggcggcaacnacaacnaccngnacaggcngnncaggaagagcaaccngaagcccnncgagagggacancagcaccgagancnaccaggccggcagcacccccngcaacggcgnggagggcnncaacngcnacnncccccngcagagcnacggcnnccagcccaccaacggcgngggcnaccagcccnacagggnggnggngcngagcnncgagcngcngcacgcccccgccaccgngngcggccccaagaagagcaccaaccnggngaagaacaagngcgngaacnnncncgagnag

SEQ ID NO: 3 - RNA, 2358 nt, synthetic construct
  source 1..2358: mol_type = other RNA
  misc_feature 1..2358: note = n is 1-methyl-3'-pseudouridylyl
anggagacagacacacnccngcnangggnacngcngcncngggnnccaggnnccacnggngaccgnacgannngggaacngaagaaagangnnnacgnggncgaacnggacnggnancccgangcgccnggcgaganggnagnncngaccngngacacncccgaagaagangggancacnnggacannggancagncaagcgaagngcnngggagnggcaaaacanngacaanacaggncaaggaannnggggacgcnggacagnacacangccacaagggcggngaggngcngncacacncacngcngnngcngcanaaaaaggaagacggaancnggncnacagacanncngaaggancagaaagaaccnaagaacaaaaccnnccngcgangcgaggcnaagaacnanncagggcggnncacgngnnggnggnngacnacnannnccaccgancngaccnncncngncaaaagcagcagaggcncancaganccccaaggcgngaccngnggcgcagcnacccngnccgccgaaagggncagaggagacaacaaggagnacgaananagcgnggagngncaggaggacagcgcangnccngccgcggaagaaagnnngccaanngaggnganggnngacgcngnncacaaacnnaagnacgagaacnacaccncnagcnncnnnancagagacancannaagcccgaccccccaaaaaancngcagcncaagccgcncaagaacagcagacaggncgaggnnncnngggagnaccccgacacanggncnacnccacacncnnannnnagncncacannnngcgngcaggngcagggnaagagnaagcgggagaaaaagganagagngnnnaccgacaaaaccncagcnacagnganangnagaaagaangcnagcancagngngcgcgcccaagaccgcnacnacagnncnnccnggncngagngggcgnccgngccnngcagcggaggcggaggcncnggaggaggcggcncnggcggaggcggancncggaaccnnccngnggcnacnccnganccnggcangnnnccnngncngcaccacagccagaacnngcngcgggcagngncnaanangcngcagaaagccaggcagacccnggagnnnnacccangnaccagcgaagaganngancangaggananaaccaaggacaagacnagcaccgnggaggcangccngccacnggagnngaccaagaacgaaagcngncncaacnccagagaaacnnccnncancacaaacggnnccngccnggcaagnagaaagaccagcnnnanganggcgcngngccngncnnccancnangaggaccncaagangnaccaggncgagnnnaagacnangaacgccaagcnccnganggacccaaagcgccagannnnnnnggancagaanangnnggccgncancgangaanngangcaggcccnnaacnnnaanagngagacngngccccagaaancaagncnggaggagccngacnncnanaagacaaagancaagcngngnannnngcnncacgcannnagganccgcgcngnaaccanagaccgagncangncnnaccngaangcnagcnncgaaggcggnggaggcagcggaggcggnggcagcggnggcggaggcagcncnagaagggngcagcccaccgagagcancgngaggnnccccaacancaccaaccngngccccnncggcgaggngnncaacgccaccaggnncgccagcgngnacgccnggaacaggaagaggancagcaacngcgnggccgacnacagcgngcngnacaacagcgccagcnncagcaccnncaagngcnacggcgngagccccaccaagcngaacgaccngngcnncaccaacgngnacgccgacagcnncgngancaggggcgacgaggngaggcagancgcccccggccagaccggcaagancgccgacnacaacnacaagcngcccgacgacnncaccggcngcgngancgccnggaacagcaacaaccnggacagcaaggngggcggcaacnacaacnaccngnacaggcngnncaggaagagcaaccngaagcccnncgagagggacancagcaccgagancnaccaggccggcagcacccccngcaacggcgnggagggcnncaacngcnacnncccccngcagagcnacggcnnccagcccaccaacggcgngggcnaccagcccnacagggnggnggngcngagcnncgagcngcngcacgcccccgccaccgngngcggccccaagaagagcaccaaccnggngaagaacaagngcgngaacnnncncgagnag

SEQ ID NO: 4 - RNA, 1218 nt, synthetic construct
  source 1..1218: mol_type = other RNA
  misc_feature 1..1218: note = n is 1-methyl-3'-pseudouridylyl
anggagacagacacacnccngcnangggnacngcngcncngggnnccaggnnccacnggngaccgnacgcacaagncaagcncacaagggcaggaccggcacangancagaangagacagnngancgacanagnngaccaacncaagaacnacgngaacgaccncgngcccgagnnncngcccgccccagaagacgnggagacgaacngngagnggnccgcanncnccngcnnccagaaggcncaacncaagagngccaanaccgggaanaangaacggancancaacgngagcannaagaagcngaaacggaaaccncccnccaccaangccgggagacggcagaaacancgcnngaccngnccancangnganncnnacgaaaagaagccncccaaggaannnnnggaacggnnnaagncnnngcnccagaaganganncaccaacaccngnccagccggacccacggcagcgagganagcnncgaaggcggnggaggcagcggaggcggnggcagcggnggcggaggcagcncnagaagggngcagcccaccgagagcancgngaggnnccccaacancaccaaccngngccccnncggcgaggngnncaacgccaccaggnncgccagcgngnacgccnggaacaggaagaggancagcaacngcgnggccgacnacagcgngcngnacaacagcgccagcnncagcaccnncaagngcnacggcgngagccccaccaagcngaacgaccngngcnncaccaacgngnacgccgacagcnncgngancaggggcgacgaggngaggcagancgcccccggccagaccggcaagancgccgacnacaacnacaagcngcccgacgacnncaccggcngcgngancgccnggaacagcaacaaccnggacagcaaggngggcggcaacnacaacnaccngnacaggcngnncaggaagagcaaccngaagcccnncgagagggacancagcaccgagancnaccaggccggcagcacccccngcaacggcgnggagggcnncaacngcnacnncccccngcagagcnacggcnnccagcccaccaacggcgngggcnaccagcccnacagggnggnggngcngagcnncgagcngcngcacgcccccgccaccgngngcggccccaagaagagcaccaaccnggngaagaacaagngcgngaacnnncncgagnag

SEQ ID NO: 5 - RNA, 1293 nt, synthetic construct
  source 1..1293: mol_type = other RNA
  misc_feature 1..1293: note = n is 1-methyl-3'-pseudouridylyl
anggagacagacacacnccngcnangggnacngcngcncngggnnccaggnnccacnggngaccgnacgnngcagganccnngnagcaanngcccagcnggcacnnnnngcgacaacaancgaaancaaancngcncaccnngcccccccaacncnnncagcncngcaggcggccagaggaccngcganancngncgccagngnaaaggggncnnnagaaccaggaaagaangnagcncnacancnaangccgagngcganngnaccccggggnnncanngccngggagcagggngcncaangngcgaacagganngcaaacaaggacaggaacngacnaagaaaggangcaaagacngcngnnncggaaccnnnaacgancagaagcggggcancngcagaccnnggaccaacngnncncnggacggaaaancngngcncgngaangggaccaaagagagggangnggngngnggacccncnccngcngaccnnagnccnggcgcgncnncngngacnccncccgcaccagcnagagagccaggccanagnccccaanncgaaggcggnggaggcagcggaggcggnggcagcggnggcggaggcagcncnagaagggngcagcccaccgagagcancgngaggnnccccaacancaccaaccngngccccnncggcgaggngnncaacgccaccaggnncgccagcgngnacgccnggaacaggaagaggancagcaacngcgnggccgacnacagcgngcngnacaacagcgccagcnncagcaccnncaagngcnacggcgngagccccaccaagcngaacgaccngngcnncaccaacgngnacgccgacagcnncgngancaggggcgacgaggngaggcagancgcccccggccagaccggcaagancgccgacnacaacnacaagcngcccgacgacnncaccggcngcgngancgccnggaacagcaacaaccnggacagcaaggngggcggcaacnacaacnaccngnacaggcngnncaggaagagcaaccngaagcccnncgagagggacancagcaccgagancnaccaggccggcagcacccccngcaacggcgnggagggcnncaacngcnacnncccccngcagagcnacggcnnccagcccaccaacggcgngggcnaccagcccnacagggnggnggngcngagcnncgagcngcngcacgcccccgccaccgngngcggccccaagaagagcaccaaccnggngaagaacaagngcgngaacnnncncgagnag

SEQ ID NO: 6 - RNA, 1362 nt, synthetic construct
  source 1..1362: mol_type = other RNA
  misc_feature 1..1362: note = n is 1-methyl-3'-pseudouridylyl
anggagacagacacacnccngcnangggnacngcngcncngggnnccaggnnccacnggngaccgnacgcngcanngngncggcganacnnacccgncnaacgancggngnngccacgagngcaggccaggcaacggganggnnagccggngnncaagancccagaacacagngngccgcccangnggaccaggannnnanaacgacgnngnnagcagcaaaccangcaaacccngcacanggngcaaccngaggagnggaagcgagcgaaagcagcncngcacagccacccaggacaccgngngnaggngncgggcaggcacacagccncnngacnccnanaaaccaggcgnnganngngcaccgngnccnccaggncannnnncnccaggcgacaancaggccngcaaacccnggacnaacngcacccnggccggcaaacanacgcngcagccngccagcaannccagcgacgccancngcgaagacagagacccnccngcnacacagccccaagaaacccagggncccccngcaagacccannacagngcagccaaccgaggccnggccnagaaccncncaggggccaagcaccagaccagnagaggngccgggcggnagagccnncgaaggcggnggaggcagcggaggcggnggcagcggnggcggaggcagcncnagaagggngcagcccaccgagagcancgngaggnnccccaacancaccaaccngngccccnncggcgaggngnncaacgccaccaggnncgccagcgngnacgccnggaacaggaagaggancagcaacngcgnggccgacnacagcgngcngnacaacagcgccagcnncagcaccnncaagngcnacggcgngagccccaccaagcngaacgaccngngcnncaccaacgngnacgccgacagcnncgngancaggggcgacgaggngaggcagancgcccccggccagaccggcaagancgccgacnacaacnacaagcngcccgacgacnncaccggcngcgngancgccnggaacagcaacaaccnggacagcaaggngggcggcaacnacaacnaccngnacaggcngnncaggaagagcaaccngaagcccnncgagagggacancagcaccgagancnaccaggccggcagcacccccngcaacggcgnggagggcnncaacngcnacnncccccngcagagcnacggcnnccagcccaccaacggcgngggcnaccagcccnacagggnggnggngcngagcnncgagcngcngcacgcccccgccaccgngngcggccccaagaagagcaccaaccnggngaagaacaagngcgngaacnnncncgagnag

SEQ ID NO: 7 - RNA, 1449 nt, synthetic construct
  source 1..1449: mol_type = other RNA
  misc_feature 1..1449: note = n is 1-methyl-3'-pseudouridylyl
anggagacagacacacnccngcnangggnacngcngcncngggnnccaggnnccacnggngaccgnacgagggngcagcccaccgagagcancgngaggnnccccaacancaccaaccngngccccnncggcgaggngnncaacgccaccaggnncgccagcgngnacgccnggaacaggaagaggancagcaacngcgnggccgacnacagcgngcngnacaacagcgccagcnncagcaccnncaagngcnacggcgngagccccaccaagcngaacgaccngngcnncaccaacgngnacgccgacagcnncgngancaggggcgacgaggngaggcagancgcccccggccagaccggcaagancgccgacnacaacnacaagcngcccgacgacnncaccggcngcgngancgccnggaacagcaacaaccnggacagcaaggngggcggcaacnacaacnaccngnacaggcngnncaggaagagcaaccngaagcccnncgagagggacancagcaccgagancnaccaggccggcagcacccccngcaacggcgnggagggcnncaacngcnacnncccccngcagagcnacggcnnccagcccaccaacggcgngggcnaccagcccnacagggnggnggngcngagcnncgagcngcngcacgcccccgccaccgngngcggccccaagaagagcaccaaccnggngaagaacaagngcgngaacnnnnncgaaggcggnggaggcagcggaggcggnggcagcggnggcggaggcagcncnagacaccgaaggcngganaaganngaagacgaaaggaaccngcacgaggacnnngnnnncangaaaacnanccagagangnaacacgggcgaaaggncccngagccngcncaacngngaggaaannaagncncaanncgagggnnnngncaagganancangcncaanaaagaggaaacgaagaaagaaaanagcnnngagangcagaaaggngaccagaacccncaganngcngcgcacgncanaagcgaggccnccncnaaaaccacaagngngcngcagngggccgaaaaaggcnacnanaccangnccaacaancnggngacacnggagaanggaaagcagcncacggncaagcgccagggacngnannanancnacgcacaggnnaccnncngnncaaaccgcgaagccncnagncaggcgccanncanngcnncccngngncngaagncnccngggcgcnncgagagaannnngcnccgcgcngccaanacgcacncaagcgccaaaccnngcgggcagcagagcanacacnngggaggagngnnngagcngcagccnggcgcnncagngnncgngaacgngaccganccnncacaggncncacacgggacaggannnacnagnnncgggcnncngaagnngcncgagnag

SEQ ID NO: 8 - RNA, 1875 nt, synthetic construct
  source 1..1875: mol_type = other RNA
  misc_feature 1..1875: note = n is 1-methyl-3'-pseudouridylyl
anggagacagacacacnccngcnangggnacngcngcncngggnnccaggnnccacnggngaccgnacggcaccngcnagancaccancnccnncaacacagccnngggaacacgnnaacgccanncaggaggcncggcgcnngcngaancngagcaggganacagccgcagagangaacgaaacagnggaagngannagngaaangnnngaccnncaagagccaacangccngcagaccagacnngagcngnacaagcaggggcngaggggancncnnacaaaacngaaagggccacnnaccanganggccncacacnanaaacagcacngcccnccaacaccngagacgnccngngcnacncagannancacnnncgagagcnnnaaagaaaancngaaggacnnncnccnggnganccccnncganngcngggagccngnccaggagnncgaaggcggnggaggcagcggaggcggnggcagcggnggcggaggcagcncnagaagggngcagcccaccgagagcancgngaggnnccccaacancaccaaccngngccccnncggcgaggngnncaacgccaccaggnncgccagcgngnacgccnggaacaggaagaggancagcaacngcgnggccgacnacagcgngcngnacaacagcgccagcnncagcaccnncaagngcnacggcgngagccccaccaagcngaacgaccngngcnncaccaacgngnacgccgacagcnncgngancaggggcgacgaggngaggcagancgcccccggccagaccggcaagancgccgacnacaacnacaagcngcccgacgacnncaccggcngcgngancgccnggaacagcaacaaccnggacagcaaggngggcggcaacnacaacnaccngnacaggcngnncaggaagagcaaccngaagcccnncgagagggacancagcaccgagancnaccaggccggcagcacccccngcaacggcgnggagggcnncaacngcnacnncccccngcagagcnacggcnnccagcccaccaacggcgngggcnaccagcccnacagggnggnggngcngagcnncgagcngcngcacgcccccgccaccgngngcggccccaagaagagcaccaaccnggngaagaacaagngcgngaacnnncncgagggcggaggngacaaaacncacacangcccaccgngcccagcaccngaacnccnggggggaccgncagncnnccncnnccccccaaaacccaaggacacccncangancncccggaccccngaggncacangcgnggnggnggacgngagccacgaagacccngaggncaagnncaacnggnacgnggacggcgnggaggngcanaangccaagacaaagccgcgggaggagcagnacaacagcacgnaccgngnggncagcgnccncaccgnccngcaccaggacnggcngaanggcaaggagnacaagngcaaggncnccaacaaagcccncccagcccccancgagaaaaccancnccaaagccaaagggcagccccgagaaccacaggngnacacccngcccccancccgggangagcngaccaagaaccaggncagccngaccngccnggncaaaggcnncnancccagcgacancgccgnggagngggagagcaangggcagccggagaacaacnacaagaccacgccncccgngcnggacnccgacggcnccnncnnccncnacagcaagcncaccgnggacaagagcaggnggcagcaggggaacgncnncncangcnccgngangcacgaggcncngcacaaccacnacacgcagaagagccncncccngncnccgggnaaanag

SEQ ID NO: 9 - RNA, 1500 nt, synthetic construct
  source 1..1500: mol_type = other RNA
  misc_feature 1..1500: note = n is 1-methyl-3'-pseudouridylyl
anggagacagacacacnccngcnangggnacngcngcncngggnnccaggnnccacnggngaccgnacggcnaaannngncgcagccnggacanngaaagcagccgcnggaagcggnagcggcagcaagcnnagggngcagcccaccgagagcancgngaggnnccccaacancaccaaccngngccccnncggcgaggngnncaacgccaccaggnncgccagcgngnacgccnggaacaggaagaggancagcaacngcgnggccgacnacagcgngcngnacaacagcgccagcnncagcaccnncaagngcnacggcgngagccccaccaagcngaacgaccngngcnncaccaacgngnacgccgacagcnncgngancaggggcgacgaggngaggcagancgcccccggccagaccggcaagancgccgacnacaacnacaagcngcccgacgacnncaccggcngcgngancgccnggaacagcaacaaccnggacagcaaggngggcggcaacnacaacnaccngnacaggcngnncaggaagagcaaccngaagcccnncgagagggacancagcaccgagancnaccaggccggcagcacccccngcaacggcgnggagggcnncaacngcnacnncccccngcagagcnacggcnnccagcccaccaacggcgngggcnaccagcccnacagggnggnggngcngagcnncgagcngcngcacgcccccgccaccgngngcggccccaagaagagcaccaaccnggngaagaacaagngcgngaacnnngaanncggcggaggngacaaaacncacacangcccaccgngcccagcaccngaacnccnggggggaccgncagncnnccncnnccccccaaaacccaaggacacccncangancncccggaccccngaggncacangcgnggnggnggacgngagccacgaagacccngaggncaagnncaacnggnacgnggacggcgnggaggngcanaangccaagacaaagccgcgggaggagcagnacaacagcacgnaccgngnggncagcgnccncaccgnccngcaccaggacnggcngaanggcaaggagnacaagngcaaggncnccaacaaagcccncccagcccccancgagaaaaccancnccaaagccaaagggcagccccgagaaccacaggngnacacccngcccccancccgggangagcngaccaagaaccaggncagccngaccngccnggncaaaggcnncnancccagcgacancgccgnggagngggagagcaangggcagccggagaacaacnacaagaccacgccncccgngcnggacnccgacggcnccnncnnccncnacagcaagcncaccgnggacaagagcaggnggcagcaggggaacgncnncncangcnccgngangcacgaggcncngcacaaccacnacacgcagaagagccncncccngncnccgggnaaanag

SEQ ID NO: 10 - RNA, 1932 nt, synthetic construct
  source 1..1932: mol_type = other RNA
  misc_feature 1..1932: note = n is 1-methyl-3'-pseudouridylyl
anggagacagacacacnccngcnangggnacngcngcncngggnnccaggnnccacnggngaccgnacggcaccngcnagancaccancnccnncaacacagccnngggaacacgnnaacgccanncaggaggcncggcgcnngcngaancngagcaggganacagccgcagagangaacgaaacagnggaagngannagngaaangnnngaccnncaagagccaacangccngcagaccagacnngagcngnacaagcaggggcngaggggancncnnacaaaacngaaagggccacnnaccanganggccncacacnanaaacagcacngcccnccaacaccngagacgnccngngcnacncagannancacnnncgagagcnnnaaagaaaancngaaggacnnncnccnggnganccccnncganngcngggagccngnccaggagnncgaaggcggnggaggcagcggaggcggnggcagcggnggcggaggcagcgcnaaannngncgcagccnggacanngaaagcagccgcnggaagcggnagcggcagcncnagaagggngcagcccaccgagagcancgngaggnnccccaacancaccaaccngngccccnncggcgaggngnncaacgccaccaggnncgccagcgngnacgccnggaacaggaagaggancagcaacngcgnggccgacnacagcgngcngnacaacagcgccagcnncagcaccnncaagngcnacggcgngagccccaccaagcngaacgaccngngcnncaccaacgngnacgccgacagcnncgngancaggggcgacgaggngaggcagancgcccccggccagaccggcaagancgccgacnacaacnacaagcngcccgacgacnncaccggcngcgngancgccnggaacagcaacaaccnggacagcaaggngggcggcaacnacaacnaccngnacaggcngnncaggaagagcaaccngaagcccnncgagagggacancagcaccgagancnaccaggccggcagcacccccngcaacggcgnggagggcnncaacngcnacnncccccngcagagcnacggcnnccagcccaccaacggcgngggcnaccagcccnacagggnggnggngcngagcnncgagcngcngcacgcccccgccaccgngngcggccccaagaagagcaccaaccnggngaagaacaagngcgngaacnnncncgagggcggaggngacaaaacncacacangcccaccgngcccagcaccngaacnccnggggggaccgncagncnnccncnnccccccaaaacccaaggacacccncangancncccggaccccngaggncacangcgnggnggnggacgngagccacgaagacccngaggncaagnncaacnggnacgnggacggcgnggaggngcanaangccaagacaaagccgcgggaggagcagnacaacagcacgnaccgngnggncagcgnccncaccgnccngcaccaggacnggcngaanggcaaggagnacaagngcaaggncnccaacaaagcccncccagcccccancgagaaaaccancnccaaagccaaagggcagccccgagaaccacaggngnacacccngcccccancccgggangagcngaccaagaaccaggncagccngaccngccnggncaaaggcnncnancccagcgacancgccgnggagngggagagcaangggcagccggagaacaacnacaagaccacgccncccgngcnggacnccgacggcnccnncnnccncnacagcaagcncaccgnggacaagagcaggnggcagcaggggaacgncnncncangcnccgngangcacgaggcncngcacaaccacnacacgcagaagagccncncccngncnccgggnaaanag